European Patent Application EP 4 230 720 A1, published August 23, 2023. Title: Strain of Rutstroemia calopus, compositions and uses. Applicant: Universidad de Almería (UAL). The sequence listing filed with the application follows.

SEQUENCE LISTING (2 sequences)

SEQ ID NO: 1 - DNA, 521 bp, Artificial Sequence
  ITS-1 Primer
cgggtagacctcccacccttgtgtatctataccatgttgctttggcaggctgctgcccccctcgggggacagccccagcgccttcgggcctgagagtcgcctgccggaggaaaaacaaactctgaactgttagtgtcgtctgagtactatattttaatagttaaaactttcaacaacggatctcttggttctggcatcgatgaagaacgcagcgaaatgcgataagtaatgtgaattgcagaattcagtgaatcatcgaatctttgaacgcacattgcgccccttggtattccggggggcatgcctgttcgagcgtcatttcaaccctcaagctcagcttggtattgggccctcgccgggtgaccggcgggccttaaagtcagtggcggcgccgttgggtcctgaacgtagtaacatacctctcgttacagggtccccgcgtgcttctgccattaaacccccaactttctatggttgacctcggatcaggtagggatacccgctgaacttaagcatatcaa

SEQ ID NO: 2 - DNA, 964 bp, Artificial Sequence
  ITS-4 Primer
cgaggtcaccatagaaagttgggggtttaatggcagaagcacgcggggaccctgtaacgagaggtatgttactacgttcaggacccaacggcgccgccactgactttaaggcccgccggtcacccggcgagggcccaataccaagctgagcttgagggttgaaatgacgctcgaacaggcatgccccccggaataccaaggggcgcaatgtgcgttcaaagattcgatgattcactgaattctgcaattcacattacttatcgcatttcgctgcgttcttcatcgatgccagaaccaagagatccgttgttgaaagttttaactattaaaatatagtactcagacgacactaacagttcagagtttgtttttcctccggcaggcgactctcaggcccgaaggcgctggggctgtcccccgaggggggcagcagcctgccaaagcaacatggtatagatacacaagggtgggaggtctacccgtgagggcatgaactctgtaatgatccttccgcaggttcccctacggaaggatcattacagagttcatgccctcacgggtagacctcccacccttgtgtatctataccatgttgctttggcaggctgctgcccccctcgggggacagccccagcgccttcgggcctgagagtcgcctgccggaggaaaaacaaactctgaactgttagtgtcgtctgagtactatattttaatagttaaaactttcaacaacggatctcttggttctggcatcgatgaagaacgcagcgaaatgcgataagtaatgtgaattgcagaattcagtgaatcatcgaatctttgaacgcacattgcgccccttggtattccggggggcatgcctgttcgagcgtcatttcaaccctcaagctcagcttggtattgggcctcgccgggtgaccggcgggccttaaagtcagtggcggcgccgttgggtcctgaacgt